European Patent Application EP 4 706 760 A2, published March 11, 2026. Title: INTEGRIN-TARGETING PROTEIN AND METHODS OF USE THEREOF. Applicant: Georgia State University Research Foundation, Inc. Application EP Divisional of EP 16 762 256.2, filed November 3, 2025. The sequence listing filed with the application follows.

SEQUENCE LISTING (3 sequences)

SEQ ID NO: 1 - protein, 105 aa, synthetic construct
  REGION 1..105: note = Segment of Wild-type CD2
KEITNALETWGALGQDINLDIPSFQMSDDIDDIKWEKTSDKKKIAQFRKEKETFKEKDTYKLFKNGTLKIKHLKTDDQDIYKVSIYDTKGKNVLEKIFDLKIQER

SEQ ID NO: 2 - protein, 105 aa, synthetic construct
  REGION 1..105: note = man-made sequence
KEITNALETWGALGQDINLDIPSFQMSDDIDDIKWEKTSDKKKIAQFRKEKETFKEKDTYKLFKNGTLKIKHLKTDDQDIYKVSIYDTKGKNVNDVCNFASRQER

SEQ ID NO: 3 - protein, 105 aa, synthetic construct
  REGION 1..105: note = Man-made Sequence
KEITNALETWGALGQDINLDIPSFQMSDDIDDIKWEKTSDKKKIAQFRKEKETFKEKDTYKLFKNGTLKIKHLKTDDQDIYKVSIYDTKGKNVLEKYDYLKIQER